European Patent Application EP 4 144 842 A1, published March 8, 2023. Title: Immobilized Enzyme,Preparation method and Use thereof. Applicant: ASYMCHEM LIFE SCIENCETIANJIN CO.,LTD. The sequence listing filed with the application follows.

SEQUENCE LISTING (15 sequences)

SEQ ID NO: 1 - protein, 459 aa, Transaminase(Chromobacterium violaceum)
  SITE (1)..(459): TA-Cv-mather line
MQKQRTTSQWRELDAAHHLHPFTDTASLNQAGARVMTRGEGVYLWDSEGNKIIDGMAGLWCVNVGYGRKDFAEAARRQMEELPFYNTFFKTTHPAVVELSSLLAEVTPAGFDRVFYTNSGSESVDTMIRMVRRYWDVQGKPEKKTLIGRWNGYHGSTIGGASLGGMKYMHEQGDLPIPGMAHIEQPWWYKHGKDMTPDEFGVVAARWLEEKILEIGADKVAAFVGEPIQGAGGVIVPPATYWPEIERICRKYDVLLVADEVICGFGRTGEWFGHQHFGFQPDLFTAAKGLSSGYLPIGAVFVGKRVAEGLIAGGDFNHGFTYSGHPVCAAVAHANVAALRDEGIVQRVKDDIGPYMQKRWRETFSRFEHVDDVRGVGMVQAFTLVKNKAKRELFPDFGEIGTLCRDIFFRNNLIMRACGDHIVSAPPLVMTRAEVDEMLAVAERCLEEFEQTLKARGLA

SEQ ID NO: 2 - protein, 459 aa, Transaminase(Chromobacterium violaceum)
  VARIANT (1)..(459): TA-Cv-V1
  MUTAGEN (1)..(459): R416T+T7C+S47C+Q380L
MQKQRTCSQWRELDAAHHLHPFTDTASLNQAGARVMTRGEGVYLWDCEGNKIIDGMAGLWCVNVGYGRKDFAEAARRQMEELPFYNTFFKTTHPAVVELSSLLAEVTPAGFDRVFYTNSGSESVDTMIRMVRRYWDVQGKPEKKTLIGRWNGYHGSTIGGASLGGMKYMHEQGDLPIPGMAHIEQPWWYKHGKDMTPDEFGVVAARWLEEKILEIGADKVAAFVGEPIQGAGGVIVPPATYWPEIERICRKYDVLLVADEVICGFGRTGEWFGHQHFGFQPDLFTAAKGLSSGYLPIGAVFVGKRVAEGLIAGGDFNHGFTYSGHPVCAAVAHANVAALRDEGIVQRVKDDIGPYMQKRWRETFSRFEHVDDVRGVGMVLAFTLVKNKAKRELFPDFGEIGTLCRDIFFRNNLIMTACGDHIVSAPPLVMTRAEVDEMLAVAERCLEEFEQTLKARGLA

SEQ ID NO: 3 - protein, 459 aa, Transaminase(Chromobacterium violaceum)
  VARIANT (1)..(459): TA-Cv-V2
  MUTAGEN (1)..(459): R416T+T7C+S47C+R405E+K90G+A95P+K304D+Q380L+I297L
MQKQRTCSQWRELDAAHHLHPFTDTASLNQAGARVMTRGEGVYLWDCEGNKIIDGMAGLWCVNVGYGRKDFAEAARRQMEELPFYNTFFGTTHPPVVELSSLLAEVTPAGFDRVFYTNSGSESVDTMIRMVRRYWDVQGKPEKKTLIGRWNGYHGSTIGGASLGGMKYMHEQGDLPIPGMAHIEQPWWYKHGKDMTPDEFGVVAARWLEEKILEIGADKVAAFVGEPIQGAGGVIVPPATYWPEIERICRKYDVLLVADEVICGFGRTGEWFGHQHFGFQPDLFTAAKGLSSGYLPLGAVFVGDRVAEGLIAGGDFNHGFTYSGHPVCAAVAHANVAALRDEGIVQRVKDDIGPYMQKRWRETFSRFEHVDDVRGVGMVLAFTLVKNKAKRELFPDFGEIGTLCEDIFFRNNLIMTACGDHIVSAPPLVMTRAEVDEMLAVAERCLEEFEQTLKARGLA

SEQ ID NO: 4 - protein, 476 aa, Transaminase(Arthrobacter citreus)
  SITE (1)..(476): TA-Ac-mather line
MGLTVQKINWEQVKEWDRKYLMRTFSTQNEYQPVPIESTEGDYLITPGGTRLLDFFNQLCCVNLGQKNQKVNAAIKEALDRYGFVWDTYATDYKAKAAKIIIEDILGDEDWPGKVRFVSTGSEAVETALNIARLYTNRPLVVTREHDYHGWTGGAATVTRLRSFRSGLVGENSESFSAQIPGSSCSSAVLMAPSSNTFQDSNGNYLKDENGELLSVKYTRRMIENYGPEQVAAVITEVSQGVGSTMPPYEYVPQIRKMTKELGVLWISDEVLTGFGRTGKWFGYQHYGVQPDIITMGKGLSSSSLPAGAVVVSKEIAAFMDKHRWESVSTYAGHPVAMAAVCANLEVMMEENLVEQAKNSGEYIRSKLELLQEKHKSIGNFDGYGLLWIVDIVNAKTKTPYVKLDRNFRHGMNPNQIPTQIIMEKALEKGVLIGGAMPNTMRIGASLNVSRGDIDKAMDALDYALDYLESGEWQQS

SEQ ID NO: 5 - protein, 476 aa, Transaminase(Arthrobacter citreus)
  VARIANT (1)..(476): TA-Ac -V1
  MUTAGEN (1)..(476): L3S+V5S+C60Y+F164L+A178L+S187A+I180V+L370A+G411D+S186G+Y384F+I389F+V252I+L404Q+E171D
MGSTSQKINWEQVKEWDRKYLMRTFSTQNEYQPVPIESTEGDYLITPGGTRLLDFFNQLYCVNLGQKNQKVNAAIKEALDRYGFVWDTYATDYKAKAAKIIIEDILGDEDWPGKVRFVSTGSEAVETALNIARLYTNRPLVVTREHDYHGWTGGAATVTRLRSLRSGLVGDNSESFSLQVPGSSCGAAVLMAPSSNTFQDSNGNYLKDENGELLSVKYTRRMIENYGPEQVAAVITEVSQGVGSTMPPYEYIPQIRKMTKELGVLWISDEVLTGFGRTGKWFGYQHYGVQPDIITMGKGLSSSSLPAGAVVVSKEIAAFMDKHRWESVSTYAGHPVAMAAVCANLEVMMEENLVEQAKNSGEYIRSKLEALQEKHKSIGNFDGFGLLWFVDIVNAKTKTPYVKQDRNFRHDMNPNQIPTQIIMEKALEKGVLIGGAMPNTMRIGASLNVSRGDIDKAMDALDYALDYLESGEWQQS

SEQ ID NO: 6 - protein, 476 aa, Transaminase(Arthrobacter citreus)
  VARIANT (1)..(476): TA-Ac -V2
  MUTAGEN (1)..(476): L3S+V5S+C60Y+F164L+A178L+S187A+I180V+L370A+G411D+S186G+Y384F+I389F+V252I+E424Q+M423K
MGSTSQKINWEQVKEWDRKYLMRTFSTQNEYQPVPIESTEGDYLITPGGTRLLDFFNQLYCVNLGQKNQKVNAAIKEALDRYGFVWDTYATDYKAKAAKIIIEDILGDEDWPGKVRFVSTGSEAVETALNIARLYTNRPLVVTREHDYHGWTGGAATVTRLRSLRSGLVGENSESFSLQVPGSSCGAAVLMAPSSNTFQDSNGNYLKDENGELLSVKYTRRMIENYGPEQVAAVITEVSQGVGSTMPPYEYIPQIRKMTKELGVLWISDEVLTGFGRTGKWFGYQHYGVQPDIITMGKGLSSSSLPAGAVVVSKEIAAFMDKHRWESVSTYAGHPVAMAAVCANLEVMMEENLVEQAKNSGEYIRSKLEALQEKHKSIGNFDGFGLLWFVDIVNAKTKTPYVKLDRNFRHDMNPNQIPTQIIKQKALEKGVLIGGAMPNTMRIGASLNVSRGDIDKAMDALDYALDYLESGEWQQS

SEQ ID NO: 7 - protein, 253 aa, Ketoreductase(Acetobacter sp. )
  SITE (1)..(253): KRED-Ac-mather line
MARVAGKVAIVSGAANGIGKATAQLLAKEGAKVVIGDLKEEDGQKAVAEIKAAGGEAAFVKLNVTDEAAWKAAIGQTLKLYGRLDIAVNNAGIAYSGSVESTSLEDWRRVQSINLDGVFLGTQVAIEAMKKSGGGSIVNLSSIEGLIGDPMLAAYNASKGGVRLFTKSAALHCAKSGYKIRVNSVHPGYIWTPMVAGLTKEDAAARQKLVDLHPIGHLGEPNDIAYGILYLASDESKFVTGSELVIDGGYTAQ

SEQ ID NO: 8 - protein, 253 aa, Ketoreductase(Acetobacter sp. )
  VARIANT (1)..(253): KRED-Ac-V1
  MUTAGEN (1)..(253): E144S+A94N+N156V
MARVAGKVAIVSGAANGIGKATAQLLAKEGAKVVIGDLKEEDGQKAVAEIKAAGGEAAFVKLNVTDEAAWKAAIGQTLKLYGRLDIAVNNAGINYSGSVESTSLEDWRRVQSINLDGVFLGTQVAIEAMKKSGGGSIVNLSSISGLIGDPMLAAYVASKGGVRLFTKSAALHCAKSGYKIRVNSVHPGYIWTPMVAGLTKEDAAARQKLVDLHPIGHLGEPNDIAYGILYLASDESKFVTGSELVIDGGYTAQ

SEQ ID NO: 9 - protein, 253 aa, Ketoreductase(Acetobacter sp. )
  VARIANT (1)..(253): KRED-Ac-V2
  MUTAGEN (1)..(253): E144S+A94T+N156T
MARVAGKVAIVSGAANGIGKATAQLLAKEGAKVVIGDLKEEDGQKAVAEIKAAGGEAAFVKLNVTDEAAWKAAIGQTLKLYGRLDIAVNNAGITYSGSVESTSLEDWRRVQSINLDGVFLGTQVAIEAMKKSGGGSIVNLSSISGLIGDPMLAAYTASKGGVRLFTKSAALHCAKSGYKIRVNSVHPGYIWTPMVAGLTKEDAAARQKLVDLHPIGHLGEPNDIAYGILYLASDESKFVTGSELVIDGGYTAQ

SEQ ID NO: 10 - protein, 541 aa, Cyclohexanone monooxygenase(Rhodococcus sp. Phi1)
  SITE (1)..(541): CHMO-Rs-mather line
MTAQISPTVVDAVVIGAGFGGIYAVHKLHNEQGLTVVGFDKADGPGGTWYWNRYPGALSDTESHLYRFSFDRDLLQDGTWKTTYITQPEILEYLESVVDRFDLRRHFRFGTEVTSAIYLEDENLWEVSTDKGEVYRAKYVVNAVGLLSAINFPDLPGLDTFEGETIHTAAWPEGKNLAGKRVGVIGTGSTGQQVITALAPEVEHLTVFVRTPQYSVPVGNRPVTKEQIDAIKADYDGIWDSVKKSAVAFGFEESTLPAMSVSEEERNRIFQEAWDHGGGFRFMFGTFGDIATDEAANEAAASFIRSKIAEIIEDPETARKLMPTGLYAKRPLCDNGYYEVYNRPNVEAVAIKENPIREVTAKGVVTEDGVLHELDVLVFATGFDAVDGNYRRIEIRGRNGLHINDHWDGQPTSYLGVTTANFPNWFMVLGPNGPFTNLPPSIETQVEWISDTVAYAERNEIRAIEPTPEAEEEWTQTCTDIANATLFTRGDSWIFGANVPGKKPSVLFYLGGLGNYRNVLAGVVADSYRGFELKSAVPVTA

SEQ ID NO: 11 - protein, 541 aa, Cyclohexanone monooxygenase(Rhodococcus sp. Phi1)
  VARIANT (1)..(541): CHMO-Rs-V1
  MUTAGEN (1)..(541): F508Y+F435N+L438A+T436S+F280V+S441V
MTAQISPTVVDAVVIGAGFGGIYAVHKLHNEQGLTVVGFDKADGPGGTWYWNRYPGALSDTESHLYRFSFDRDLLQDGTWKTTYITQPEILEYLESVVDRFDLRRHFRFGTEVTSAIYLEDENLWEVSTDKGEVYRAKYVVNAVGLLSAINFPDLPGLDTFEGETIHTAAWPEGKNLAGKRVGVIGTGSTGQQVITALAPEVEHLTVFVRTPQYSVPVGNRPVTKEQIDAIKADYDGIWDSVKKSAVAFGFEESTLPAMSVSEEERNRIFQEAWDHGGGVRFMFGTFGDIATDEAANEAAASFIRSKIAEIIEDPETARKLMPTGLYAKRPLCDNGYYEVYNRPNVEAVAIKENPIREVTAKGVVTEDGVLHELDVLVFATGFDAVDGNYRRIEIRGRNGLHINDHWDGQPTSYLGVTTANFPNWFMVLGPNGPNSNAPPVIETQVEWISDTVAYAERNEIRAIEPTPEAEEEWTQTCTDIANATLFTRGDSWIFGANVPGKKPSVLYYLGGLGNYRNVLAGVVADSYRGFELKSAVPVTA

SEQ ID NO: 12 - protein, 541 aa, Cyclohexanone monooxygenase(Rhodococcus sp. Phi1)
  VARIANT (1)..(541): CHMO-Rs-V2
  MUTAGEN (1)..(541): F508Y+F435N+L438A+T436S+F280V+S441V+L510V
MTAQISPTVVDAVVIGAGFGGIYAVHKLHNEQGLTVVGFDKADGPGGTWYWNRYPGALSDTESHLYRFSFDRDLLQDGTWKTTYITQPEILEYLESVVDRFDLRRHFRFGTEVTSAIYLEDENLWEVSTDKGEVYRAKYVVNAVGLLSAINFPDLPGLDTFEGETIHTAAWPEGKNLAGKRVGVIGTGSTGQQVITALAPEVEHLTVFVRTPQYSVPVGNRPVTKEQIDAIKADYDGIWDSVKKSAVAFGFEESTLPAMSVSEEERNRIFQEAWDHGGGVRFMFGTFGDIATDEAANEAAASFIRSKIAEIIEDPETARKLMPTGLYAKRPLCDNGYYEVYNRPNVEAVAIKENPIREVTAKGVVTEDGVLHELDVLVFATGFDAVDGNYRRIEIRGRNGLHINDHWDGQPTSYLGVTTANFPNWFMVLGPNGPNSNAPPVIETQVEWISDTVAYAERNEIRAIEPTPEAEEEWTQTCTDIANATLFTRGDSWIFGANVPGKKPSVLYYVGGLGNYRNVLAGVVADSYRGFELKSAVPVTA

SEQ ID NO: 13 - protein, 603 aa, Cyclohexanone monooxygenase(Rhodococcus ruber-SD1)
  SITE (1)..(603): CHMO-Rr-mather line
MTTSIDREALRRKYAEERDKRIRPDGNDQYIRLDHVDGWSHDPYMPITPREPKLDHVTFAFIGGGFSGLVTAARLRESGVESVRIIDKAGDFGGVWYWNRYPGAMCDTAAMVYMPLLEETGYMPTEKYAHGPEILEHCQRIGKHYDLYDDALFHTEVTDLVWQEHDQRWRISTNRGDHFTAQFVGMGTGPLHVAQLPGIPGIESFRGKSFHTSRWDYDYTGGDALGAPMDKLADKRVAVIGTGATAVQCVPELAKYCRELYVVQRTPSAVDERGNHPIDEKWFAQIATPGWQKRWLDSFTAIWDGVLTDPSELAIEHEDLVQDGWTALGQRMRAAVGSVPIEQYSPENVQRALEEADDEQMERIRARVDEIVTDPATAAQLKAWFRQMCKRPCFHDDYLPAFNRPNTHLVDTGGKGVERITENGVVVAGVEYEVDCIVYASGFEFLGTGYTDRAGFDPTGRDGVKLSEHWAQGTRTLHGMHTYGFPNLFVLQLMQGAALGSNIPHNFVEAARVVAAIVDHVLSTGTSSVETTKEAEQAWVQLLLDHGRPLGNPECTPGYYNNEGKPAELKDRLNVGYPAGSAAFFRMMDHWLAAGSFDGLTFR

SEQ ID NO: 14 - protein, 603 aa, Cyclohexanone monooxygenase(Rhodococcus ruber-SD1)
  VARIANT (1)..(603): CHMO-Rr-V1
  MUTAGEN (1)..(603): P190L+Y559M+C249V+C393V+C257A+M45T
MTTSIDREALRRKYAEERDKRIRPDGNDQYIRLDHVDGWSHDPYTPITPREPKLDHVTFAFIGGGFSGLVTAARLRESGVESVRIIDKAGDFGGVWYWNRYPGAMCDTAAMVYMPLLEETGYMPTEKYAHGPEILEHCQRIGKHYDLYDDALFHTEVTDLVWQEHDQRWRISTNRGDHFTAQFVGMGTGLLHVAQLPGIPGIESFRGKSFHTSRWDYDYTGGDALGAPMDKLADKRVAVIGTGATAVQVVPELAKYARELYVVQRTPSAVDERGNHPIDEKWFAQIATPGWQKRWLDSFTAIWDGVLTDPSELAIEHEDLVQDGWTALGQRMRAAVGSVPIEQYSPENVQRALEEADDEQMERIRARVDEIVTDPATAAQLKAWFRQMCKRPVFHDDYLPAFNRPNTHLVDTGGKGVERITENGVVVAGVEYEVDCIVYASGFEFLGTGYTDRAGFDPTGRDGVKLSEHWAQGTRTLHGMHTYGFPNLFVLQLMQGAALGSNIPHNFVEAARVVAAIVDHVLSTGTSSVETTKEAEQAWVQLLLDHGRPLGNPECTPGMYNNEGKPAELKDRLNVGYPAGSAAFFRMMDHWLAAGSFDGLTFR

SEQ ID NO: 15 - protein, 603 aa, Cyclohexanone monooxygenase(Rhodococcus ruber-SD1)
  VARIANT (1)..(603): CHMO-Rr-V2
  MUTAGEN (1)..(603): Y559M+P190L+P504V
MTTSIDREALRRKYAEERDKRIRPDGNDQYIRLDHVDGWSHDPYMPITPREPKLDHVTFAFIGGGFSGLVTAARLRESGVESVRIIDKAGDFGGVWYWNRYPGAMCDTAAMVYMPLLEETGYMPTEKYAHGPEILEHCQRIGKHYDLYDDALFHTEVTDLVWQEHDQRWRISTNRGDHFTAQFVGMGTGLLHVAQLPGIPGIESFRGKSFHTSRWDYDYTGGDALGAPMDKLADKRVAVIGTGATAVQCVPELAKYCRELYVVQRTPSAVDERGNHPIDEKWFAQIATPGWQKRWLDSFTAIWDGVLTDPSELAIEHEDLVQDGWTALGQRMRAAVGSVPIEQYSPENVQRALEEADDEQMERIRARVDEIVTDPATAAQLKAWFRQMCKRPCFHDDYLPAFNRPNTHLVDTGGKGVERITENGVVVAGVEYEVDCIVYASGFEFLGTGYTDRAGFDPTGRDGVKLSEHWAQGTRTLHGMHTYGFPNLFVLQLMQGAALGSNIVHNFVEAARVVAAIVDHVLSTGTSSVETTKEAEQAWVQLLLDHGRPLGNPECTPGMYNNEGKPAELKDRLNVGYPAGSAAFFRMMDHWLAAGSFDGLTFR